European Patent Specification EP 3 461 492 B1, published April 30, 2025. Title: COMPOSITIONS AND METHODS FOR THE TREATMENT OF CARBOXYHEMOGLOBINEMIA. Applicant: UNIVERSITY OF PITTSBURGH - OF THE COMMONWEALTH SYSTEM OF HIGHER EDUCATION. Application EP. The sequence listing filed with the application follows.

SEQUENCE LISTING (6 sequences)

SEQ ID NO: 1 - protein, 151 aa, Homo sapiens
MERPEPELIRQSWRAVSRSPLEHGTVLFARLFALEPDLLPLFQYNCRQFSSPEDCLSSPEFLDHIRKVMLVIDAAVTNVEDLSSLEEYLASLGRKHRAVGVKLSSFSTVGESLLYMLEKCLGPAFTPATRAAWSQLYGAVVQAMSRGWDGE

SEQ ID NO: 2 - protein, 151 aa, Artificial Sequence
  Recombinant polypeptide
  MISC_FEATURE (46)..(46): Xaa = Cys or Gly
  MISC_FEATURE (55)..(55): Xaa = Cys or Ser
  MISC_FEATURE (64)..(64): Xaa = Gln, Leu, Ala, Trp
  MISC_FEATURE (120)..(120): Xaa = Cys or Ser
MERPEPELIRQSWRAVSRSPLEHGTVLFARLFALEPDLLPLFQYNXRQFSSPEDXLSSPEFLDXIRKVMLVIDAAVTNVEDLSSLEEYLASLGRKHRAVGVKLSSFSTVGESLLYMLEKXLGPAFTPATRAAWSQLYGAVVQAMSRGWDGE

SEQ ID NO: 3 - protein, 151 aa, Artificial Sequence
  Recombinant polypeptide
MERPEPELIRQSWRAVSRSPLEHGTVLFARLFALEPDLLPLFQYNGRQFSSPEDSLSSPEFLDQIRKVMLVIDAAVTNVEDLSSLEEYLASLGRKHRAVGVKLSSFSTVGESLLYMLEKSLGPAFTPATRAAWSQLYGAVVQAMSRGWDGE

SEQ ID NO: 4 - protein, 190 aa, Homo sapiens
MEKVPGEMEIERRERSEELSEAERKAVQAMWARLYANCEDVGVAILVRFFVNFPSAKQYFSQFKHMEDPLEMERSPQLRKHACRVMGALNTVVENLHDPDKVSSVLALVGKAHALKHKVEPVYFKILSGVILEVVAEEFASDFPPETQRAWAKLRGLIYSHVTAAYKEVGWVQQVPNATTPPATLPSSGP

SEQ ID NO: 5 - protein, 190 aa, Artificial Sequence
  Recombinant polypeptide
  MISC_FEATURE (38)..(38): Xaa = Cys or Ser
  MISC_FEATURE (81)..(81): Xaa = Gln, Leu, Ala or Trp
  MISC_FEATURE (83)..(83): Xaa = Cys or Ser
MEKVPGEMEIERRERSEELSEAERKAVQAMWARLYANXEDVGVAILVRFFVNFPSAKQYFSQFKHMEDPLEMERSPQLRKXAXRVMGALNTVVENLHDPDKVSSVLALVGKAHALKHKVEPVYFKILSGVILEVVAEEFASDFPPETQRAWAKLRGLIYSHVTAAYKEVGWVQQVPNATTPPATLPSSGP

SEQ ID NO: 6 - protein, 190 aa, Artificial Sequence
  Recombinant polypeptide
MEKVPGEMEIERRERSEELSEAERKAVQAMWARLYANSEDVGVAILVRFFVNFPSAKQYFSQFKHMEDPLEMERSPQLRKQASRVMGALNTVVENLHDPDKVSSVLALVGKAHALKHKVEPVYFKILSGVILEVVAEEFASDFPPETQRAWAKLRGLIYSHVTAAYKEVGWVQQVPNATTPPATLPSSGP